European Patent Application EP 4 703 375 A1, published March 4, 2026. Title: 一种T细胞受体及其用途. Applicant: 苏州沙砾生物科技有限公司. Application WO. The sequence listing filed with the application follows.

SEQUENCE LISTING (41 sequences)

SEQ ID NO: 1 - protein, 133 aa, synthetic construct
MTIRLLCYMGFYFLGAGLMEADIYQTPRYLVIGTGKKITLECSQTMGHDKMYWYQQDPGMELHLIHYSYGVNSTEKGDLSSESTVSRIRTEHFPLTLESARPSHTSQYLCASSDRQGAQEQYFGPGTRLTVTE

SEQ ID NO: 2 - protein, 135 aa, synthetic construct
MTIRLLCYMGFYFLGAGLMEADIYQTPRYLVIGTGKKITLECSQTMGHDKMYWYQQDPGMELHLIHYSYGVNSTEKGDLSSESTVSRIRTEHFPLTLESARPSHTSQYLCASSDTNQVQVHEQFFGPGTRLTVLE

SEQ ID NO: 3 - protein, 134 aa, synthetic construct
MTIRLLCYMGFYFLGAGLMEADIYQTPRYLVIGTGKKITLECSQTMGHDKMYWYQQDPGMELHLIHYSYGVNSTEKGDLSSESTVSRIRTEHFPLTLESARPSHTSQYLCASSLRTGEGNEQFFGPGTRLTVLE

SEQ ID NO: 4 - protein, 137 aa, synthetic construct
MTIRLLCYMGFYFLGAGLMEADIYQTPRYLVIGTGKKITLECSQTMGHDKMYWYQQDPGMELHLIHYSYGVNSTEKGDLSSESTVSRIRTEHFPLTLESARPSHTSQYLCASSEPTGLAGGADTQYFGPGTRLTVLE

SEQ ID NO: 5 - protein, 132 aa, synthetic construct
MTIRLLCYMGFYFLGAGLMEADIYQTPRYLVIGTGKKITLECSQTMGHDKMYWYQQDPGMELHLIHYSYGVNSTEKGDLSSESTVSRIRTEHFPLTLESARPSHTSQYLCASSEDRAHEQYFGPGTRLTVTE

SEQ ID NO: 6 - protein, 134 aa, synthetic construct
MTIRLLCYMGFYFLGAGLMEADIYQTPRYLVIGTGKKITLECSQTMGHDKMYWYQQDPGMELHLIHYSYGVNSTEKGDLSSESTVSRIRTEHFPLTLESARPSHTSQYLCASSESLGTTYEQYFGPGTRLTVTE

SEQ ID NO: 7 - protein, 133 aa, synthetic construct
MTIRLLCYMGFYFLGAGLMEADIYQTPRYLVIGTGKKITLECSQTMGHDKMYWYQQDPGMELHLIHYSYGVNSTEKGDLSSESTVSRIRTEHFPLTLESARPSHTSQYLCASSEKAGKYEQYFGPGTRLTVTE

SEQ ID NO: 8 - protein, 136 aa, synthetic construct
MTIRLLCYMGFYFLGAGLMEADIYQTPRYLVIGTGKKITLECSQTMGHDKMYWYQQDPGMELHLIHYSYGVNSTEKGDLSSESTVSRIRTEHFPLTLESARPSHTSQYLCASSPPSVQGARYEQYFGPGTRLTVTE

SEQ ID NO: 9 - protein, 135 aa, synthetic construct
MTIRLLCYMGFYFLGAGLMEADIYQTPRYLVIGTGKKITLECSQTMGHDKMYWYQQDPGMELHLIHYSYGVNSTEKGDLSSESTVSRIRTEHFPLTLESARPSHTSQYLCASSGSQGISYNEQFFGPGTRLTVLE

SEQ ID NO: 10 - protein, 134 aa, synthetic construct
MTIRLLCYMGFYFLGAGLMEADIYQTPRYLVIGTGKKITLECSQTMGHDKMYWYQQDPGMELHLIHYSYGVNSTEKGDLSSESTVSRIRTEHFPLTLESARPSHTSQYLCASSENRGGNQPQHFGDGTRLSILE

SEQ ID NO: 11 - protein, 135 aa, synthetic construct
MTIRLLCYMGFYFLGAGLMEADIYQTPRYLVIGTGKKITLECSQTMGHDKMYWYQQDPGMELHLIHYSYGVNSTEKGDLSSESTVSRIRTEHFPLTLESARPSHTSQYLCASSDTWKGANEKLFFGSGTQLSVLE

SEQ ID NO: 12 - protein, 135 aa, synthetic construct
MTIRLLCYMGFYFLGAGLMEADIYQTPRYLVIGTGKKITLECSQTMGHDKMYWYQQDPGMELHLIHYSYGVNSTEKGDLSSESTVSRIRTEHFPLTLESARPSHTSQYLCASSEPIQGAQYEQYFGPGTRLTVTE

SEQ ID NO: 13 - protein, 133 aa, synthetic construct
MTIRLLCYMGFYFLGAGLMEADIYQTPRYLVIGTGKKITLECSQTMGHDKMYWYQQDPGMELHLIHYSYGVNSTEKGDLSSESTVSRIRTEHFPLTLESARPSHTSQYLCASTSTGPYNEQFFGPGTRLTVLE

SEQ ID NO: 14 - protein, 10 aa, synthetic construct
SDRQGAQEQY

SEQ ID NO: 15 - protein, 12 aa, synthetic construct
SDTNQVQVHEQF

SEQ ID NO: 16 - protein, 11 aa, synthetic construct
SLRTGEGNEQF

SEQ ID NO: 17 - protein, 14 aa, synthetic construct
SEPTGLAGGADTQY

SEQ ID NO: 18 - protein, 9 aa, synthetic construct
SEDRAHEQY

SEQ ID NO: 19 - protein, 11 aa, synthetic construct
SESLGTTYEQY

SEQ ID NO: 20 - protein, 10 aa, synthetic construct
SEKAGKYEQY

SEQ ID NO: 21 - protein, 13 aa, synthetic construct
SPPSVQGARYEQY

SEQ ID NO: 22 - protein, 12 aa, synthetic construct
SGSQGISYNEQF

SEQ ID NO: 23 - protein, 11 aa, synthetic construct
SENRGGNQPQH

SEQ ID NO: 24 - protein, 12 aa, synthetic construct
SDTWKGANEKLF

SEQ ID NO: 25 - protein, 12 aa, synthetic construct
SEPIQGAQYEQY

SEQ ID NO: 26 - protein, 10 aa, synthetic construct
TSTGPYNEQF

SEQ ID NO: 27 - protein, 15 aa, synthetic construct
IHYSYGVNSTEKGDL

SEQ ID NO: 28 - protein, 8 aa, synthetic construct
QTMGHDKM

SEQ ID NO: 29 - protein, 176 aa, synthetic construct
DLKNVFPPEVAVFEPSEAEISHTQKATLVCLATGFFPDHVELSWWVNGKEVHSGVSTDPQPLKEQPALNDSRYCLSSRLRVSATFWQNPRNHFRCQVQFYGLSENDEWTQDRAKPVTQIVSAEAWGRADCGFTSVSYQQGVLSATILYEILLGKATLYAVLVSALVLMAMVKRKDF

SEQ ID NO: 30 - protein, 176 aa, synthetic construct
DLNKVFPPEVAVFEPSEAEISHTQKATLVCLATGFFPDHVELSWWVNGKEVHSGVSTDPQPLKEQPALNDSRYCLSSRLRVSATFWQNPRNHFRCQVQFYGLSENDEWTQDRAKPVTQIVSAEAWGRADCGFTSVSYQQGVLSATILYEILLGKATLYAVLVSALVLMAMVKRKDF

SEQ ID NO: 31 - protein, 15 aa, synthetic construct
CVVSDRGSTLGRLYF

SEQ ID NO: 32 - protein, 7 aa, synthetic construct
MTFSENT

SEQ ID NO: 33 - protein, 6 aa, synthetic construct
VSPFSN

SEQ ID NO: 34 - protein, 135 aa, synthetic construct
MKKHLTTFLVILWLYFYRGNGKNQVEQSPQSLIILEGKNCTLQCNYTVSPFSNLRWYKQDTGRGPVSLTIMTFSENTKSNGRYTATLDADTKQSSLHITASQLSDSASYICVVSDRGSTLGRLYFGRGTQLTVWP

SEQ ID NO: 35 - protein, 141 aa, synthetic construct
DIQNPDPAVYQLRDSKSSDKSVCLFTDFDSQTNVSQSKDSDVYITDKTVLDMRSMDFKSNSAVAWSNKSDFACANAFNNSIIPEDTFFPSPESSCDVKLVEKSFETDTNLNFQNLSVIGFRILLLKVAGFNLLMTLRLWSS

SEQ ID NO: 36 - protein, 276 aa, synthetic construct
MKKHLTTFLVILWLYFYRGNGKNQVEQSPQSLIILEGKNCTLQCNYTVSPFSNLRWYKQDTGRGPVSLTIMTFSENTKSNGRYTATLDADTKQSSLHITASQLSDSASYICVVSDRGSTLGRLYFGRGTQLTVWPDIQNPDPAVYQLRDSKSSDKSVCLFTDFDSQTNVSQSKDSDVYITDKTVLDMRSMDFKSNSAVAWSNKSDFACANAFNNSIIPEDTFFPSPESSCDVKLVEKSFETDTNLNFQNLSVIGFRILLLKVAGFNLLMTLRLWSS

SEQ ID NO: 37 - protein, 313 aa, synthetic construct
MTIRLLCYMGFYFLGAGLMEADIYQTPRYLVIGTGKKITLECSQTMGHDKMYWYQQDPGMELHLIHYSYGVNSTEKGDLSSESTVSRIRTEHFPLTLESARPSHTSQYLCASSEGGGLKLAKNIQYFGAGTRLSVLEDLNKVFPPEVAVFEPSEAEISHTQKATLVCLATGFFPDHVELSWWVNGKEVHSGVSTDPQPLKEQPALNDSRYCLSSRLRVSATFWQNPRNHFRCQVQFYGLSENDEWTQDRAKPVTQIVSAEAWGRADCGFTSVSYQQGVLSATILYEILLGKATLYAVLVSALVLMAMVKRKDF

SEQ ID NO: 38 - protein, 276 aa, synthetic construct; identical to SEQ ID NO: 36

SEQ ID NO: 39 - protein, 134 aa, synthetic construct
MGFRLLCCVAFCLLGAGPVDSGVTQTPKHLITATGQRVTLRCSPRSGDLSVYWYQQSLDQGLQFLIQYYNGEERAKGNILERFSAQQFPDLHSELNLSSLELGDSALYFCASSARDWIYNEQFFGPGTRLTVLE

SEQ ID NO: 40 - protein, 136 aa, synthetic construct
MTIRLLCYVGFYFLGAGLMEADIYQTPRYLVIGTGKKITLECSQTMGHDKMYWYQQDPGMELHLIHYSYGVNSTEKGDLSSESTVSRIRTEHFPLTLESARPSHTSQYLCASSPSLAAPSNYGYTFGSGTRLTVVE

SEQ ID NO: 41 - protein, 135 aa, synthetic construct
MMKCPQALLAIFWLLLSWVSSEDKVVQSPLSLVVHEGDTVTLNCSYEVTNFRSLLWYKQEKKAPTFLFMLTSSGIEKKSGRLSSILDKKELFSILNITATQTGDSAVYLCAVEGDSGGGADGLTFGKGTHLIIQP